European Patent Specification EP 3 494 989 B1, published July 16, 2025. Title: COMPOSITE ANTIGENIC SEQUENCES AND VACCINES. Applicant: LONGHORN VACCINES AND DIAGNOSTICS, LLC. Application PCT/US2013/023269. The sequence listing filed with the application follows.

SEQUENCE LISTING (115 sequences)

SEQ ID NO: 1 - protein, 19 aa, Influenza virus
DWSGYSGSFVQHPELTGLD

SEQ ID NO: 2 - protein, 7 aa, Influenza virus
ETPIRNE

SEQ ID NO: 3 - protein, 15 aa, Influenza virus
FVIREPFISCSHLEC

SEQ ID NO: 4 - protein, 6 aa, Influenza virus
GNFIAP

SEQ ID NO: 5 - protein, 6 aa, Influenza virus
GNLIAP

SEQ ID NO: 6 - protein, 7 aa, Influenza virus
GNLFIAP

SEQ ID NO: 7 - protein, 7 aa, Influenza virus
GNLIFAP

SEQ ID NO: 8 - protein, 8 aa, Influenza virus
HYEECSCY

SEQ ID NO: 9 - protein, 10 aa, Influenza virus
LLTEVETPIR

SEQ ID NO: 10 - protein, 11 aa, Influenza virus
LLTEVETPIRN

SEQ ID NO: 11 - protein, 12 aa, Influenza virus
LLTEVETPIRNE

SEQ ID NO: 12 - protein, 18 aa, Influenza virus
DWSGYSGSFVQHPELTGL

SEQ ID NO: 13 - protein, 9 aa, Influenza virus
EVETPIRNE

SEQ ID NO: 14 - protein, 38 aa, Influenza virus
FLLPEDETPIRNEWGLLTDDETPIRYIKANSKFIGITE

SEQ ID NO: 15 - protein, 64 aa, Influenza virus
GNLFIAPGNLFIAPHYEECSCYHYEECSCYQYIKANSKFIGITEHYEECSCYTPIRNETPIRNE

SEQ ID NO: 16 - protein, 35 aa, Influenza virus
GNLFIAPGNLFIAPQYIKANSKFIGITEGNLFIAP

SEQ ID NO: 17 - protein, 48 aa, Influenza virus
HYEECSCYDWSGYSGSFVQHPELTGLHYEECSCYQYIKANSKFIGITE

SEQ ID NO: 18 - protein, 33 aa, Influenza virus
ITGFAPFSKDNSIRLSAGGDIWVTREPYVSCDP

SEQ ID NO: 19 - protein, 7 aa, Influenza virus
IWGIHHP

SEQ ID NO: 20 - protein, 7 aa, Influenza virus
IWGVHHP

SEQ ID NO: 21 - protein, 8 aa, Influenza virus
IWGVIHHP

SEQ ID NO: 22 - protein, 8 aa, Influenza virus
IWGIVHHP

SEQ ID NO: 23 - protein, 16 aa, Influenza virus
KSCINRCFYVELIRGR

SEQ ID NO: 24 - protein, 27 aa, Influenza virus
LLTEVETPIRNESLLTEVETPIRNEWG

SEQ ID NO: 25 - protein, 13 aa, Influenza virus
LLTEVETPIRNEW

SEQ ID NO: 26 - protein, 14 aa, Influenza virus
LLTEVETPIRNEWG

SEQ ID NO: 27 - protein, 11 aa, Influenza virus
LTEVETPIRNE

SEQ ID NO: 28 - protein, 12 aa, Influenza virus
LTEVETPIRNEW

SEQ ID NO: 29 - protein, 13 aa, Influenza virus
LTEVETPIRNEWG

SEQ ID NO: 30 - protein, 9 aa, Influenza virus
MSLLTEVET

SEQ ID NO: 31 - protein, 10 aa, Influenza virus
MSLLTEVETP

SEQ ID NO: 32 - protein, 11 aa, Influenza virus
MSLLTEVETPI

SEQ ID NO: 33 - protein, 12 aa, Influenza virus
MSLLTEVETPIR

SEQ ID NO: 34 - protein, 13 aa, Influenza virus
MSLLTEVETPIRN

SEQ ID NO: 35 - protein, 14 aa, Influenza virus
MSLLTEVETPIRNE

SEQ ID NO: 36 - protein, 20 aa, Influenza virus
MSLLTEVETPIRNETPIRNE

SEQ ID NO: 37 - protein, 15 aa, Influenza virus
MSLLTEVETPIRNEW

SEQ ID NO: 38 - protein, 16 aa, Influenza virus
MSLLTEVETPIRNEWG

SEQ ID NO: 39 - protein, 24 aa, Influenza virus
MSLLTEVETPIRNEWGCRCNDSSD

SEQ ID NO: 40 - protein, 8 aa, Influenza virus
SLLTEVET

SEQ ID NO: 41 - protein, 13 aa, Influenza virus
SLLTEVETPIRNE

SEQ ID NO: 42 - protein, 14 aa, Influenza virus
SLLTEVETPIRNEW

SEQ ID NO: 43 - protein, 15 aa, Influenza virus
SLLTEVETPIRNEWG

SEQ ID NO: 44 - protein, 21 aa, Influenza virus
SLLTEVETPIRNEWGTPIRNE

SEQ ID NO: 45 - protein, 27 aa, Influenza virus
SLLTEVETPIRNEWGTPIRNETPIRNE

SEQ ID NO: 46 - protein, 33 aa, Influenza virus
SLLTEVETPIRNEWGTPIRNETPIRNETPIRNE

SEQ ID NO: 47 - protein, 39 aa, Influenza virus
SLLTEVETPIRNEWGLLTEVETPIRQYIKANSKFIGITE

SEQ ID NO: 48 - protein, 10 aa, Influenza virus
TEVETPIRNE

SEQ ID NO: 49 - protein, 6 aa, Influenza virus
TPIRNE

SEQ ID NO: 50 - protein, 8 aa, Influenza virus
VETPIRNE

SEQ ID NO: 51 - protein, 52 aa, Influenza virus
VTREPYVSCDPKSCINRCFYVELIRGRVTREPYVSCDPWYIKANSKFIGITE

SEQ ID NO: 52 - protein, 6 aa, Influenza virus
WGIHHP

SEQ ID NO: 53 - protein, 6 aa, Influenza virus
WGVHHP

SEQ ID NO: 54 - protein, 7 aa, Influenza virus
WGVIHHP

SEQ ID NO: 55 - protein, 7 aa, Influenza virus
WGIVHHP

SEQ ID NO: 56 - protein, 8 aa, Influenza virus
YIWGIHHP

SEQ ID NO: 57 - protein, 8 aa, Influenza virus
YIWGVHHP

SEQ ID NO: 58 - protein, 9 aa, Influenza virus
YIWGVIHHP

SEQ ID NO: 59 - protein, 9 aa, Influenza virus
YIWGIVHHP

SEQ ID NO: 60 - protein, 14 aa, Influenza virus
QYIKANSKFIGITE

SEQ ID NO: 61 - protein, 15 aa, Influenza virus
PIRNEWGCRCNDSSD

SEQ ID NO: 62-64 - skipped (3 entries)

SEQ ID NO: 65 - protein, 372 aa, Artificial Sequence
  Description of Artificial Sequence: Synthetic polypeptide
SEYAYGSFVRTVSLPVGADEGNLFIAPWGVIHHPHYEECSCYGLPVEYLQVPSPSMGRDIKVQFQSGGANSPALYLLDGLRAQDDFSGWDINTPAFEWYDQSGLSVVMPVGGQSSFYSDWYQPACRKAGCQTYKWETFLTSELPGWLQANRHVQPTGSAVVGLSMAASSALTLAIYHPQQFVYAGAMSGLLDPSQAMGPTLIGLAMGDAGGYKASDMWGPKEDPAWQRNDPLLNVGKLIANNTRVWVYCGNGKPSDLGGNNLPAKFLEGFVRTSNIKFQDAYNAGGHNGVFDFPDSGTHSWEYWGAQLNAMKPDLQRHWVPRPTPGPPQGAFDFPDSGTHSWEYWGAQLNAMKPDLQRHWVPRPTPGPPQGA

SEQ ID NO: 66 - protein, 22 aa, Artificial Sequence
  Description of Artificial Sequence: Synthetic peptide
GNLFIAPWGVIHHPHYEECSCY

SEQ ID NO: 67 - protein, 22 aa, Artificial Sequence
  Description of Artificial Sequence: Synthetic peptide
WGVIHHPGNLFIAPHYEECSCY

SEQ ID NO: 68 - protein, 294 aa, Mycobacterium tuberculosis
SRPGLPVEYLQVPSPSMGRDIKVQFQSGGANSPALYLLDGLRAQDDFSGWDINTPAFEWYDQSGLSVVMPVGGQSSFYSDWYQPACGKAGCQTYKWETFLTSELPGWLQANRHVKPTGSAVVGLSMAASSALTLAIYHPQQFVYAGAMSGLLDPSQAMGPTLIGLAMGDAGGYKASDMWGPKEDPAWQRNDPLLNVGKLIANNTRVWVYCGNGKPSDLGGNNLPAKFLEGFVRTSNIKFQDAYNAGGGHNGVFDFPDSGTHSWEYWGAQLNAMKPDLQRALGATPNTGPAPQGA

SEQ ID NO: 69 - DNA, 882 bp, Mycobacterium tuberculosis
tcccggccgggcttgccggtggagtacctgcaggtgccgtcgccgtcgatgggccgtgacatcaaggtccaattccaaagtggtggtgccaactcgcccgccctgtacctgctcgacggcctgcgcgcgcaggacgacttcagcggctgggacatcaacaccccggcgttcgagtggtacgaccagtcgggcctgtcggtggtcatgccggtgggtggccagtcaagcttctactccgactggtaccagcccgcctgcggcaaggccggttgccagacttacaagtgggagaccttcctgaccagcgagctgccggggtggctgcaggccaacaggcacgtcaagcccaccggaagcgccgtcgtcggtctttcgatggctgcttcttcggcgctgacgctggcgatctatcacccccagcagttcgtctacgcgggagcgatgtcgggcctgttggacccctcccaggcgatgggtcccaccctgatcggcctggcgatgggtgacgctggcggctacaaggcctccgacatgtggggcccgaaggaggacccggcgtggcagcgcaacgacccgctgttgaacgtcgggaagctgatcgccaacaacacccgcgtctgggtgtactgcggcaacggcaagccgtcggatctgggtggcaacaacctgccggccaagttcctcgagggcttcgtgcggaccagcaacatcaagttccaagacgcctacaacgccggtggcggccacaacggcgtgttcgacttcccggacagcggtacgcacagctgggagtactggggcgcgcagctcaacgctatgaagcccgacctgcaacgggcactgggtgccacgcccaacaccgggcccgcgccccagggcgcc

SEQ ID NO: 70 - protein, 336 aa, Artificial Sequence
  Description of Artificial Sequence: Synthetic polypeptide
SEFAYGSFVRTVSLPVGADEGNLFIAPWGVIHHPHYEECSCYSRPGLPVEYLQVPSPSMGRDIKVQFQSGGANSPALYLLDGLRAQDDFSGWDINTPAFEWYDQSGLSVVMPVGGQSSFYSDWYQPACGKAGCQTYKWETFLTSELPGWLQANRHVKPTGSAVVGLSMAASSALTLAIYHPQQFVYAGAMSGLLDPSQAMGPTLIGLAMGDAGGYKASDMWGPKEDPAWQRNDPLLNVGKLIANNTRVWVYCGNGKPSDLGGNNLPAKFLEGFVRTSNIKFQDAYNAGGGHNGVFDFPDSGTHSWEYWGAQLNAMKPDLQRALGATPNTGPAPQGA

SEQ ID NO: 71 - DNA, 1038 bp, Artificial Sequence
  Description of Artificial Sequence: Synthetic polynucleotide
tttgggcccattatgtcggaattcgcgtacggttccttcgttcgcacggtgtcgctgccggtaggtgctgacgaggggaatctattcattgctccttggggggttattcaccacccgcattatgaggaatgttcctgttactcccggccgggcttgccggtggagtacctgcaggtgccgtcgccgtcgatgggccgtgacatcaaggtccaattccaaagtggtggtgccaactcgcccgccctgtacctgctcgacggcctgcgcgcgcaggacgacttcagcggctgggacatcaacaccccggcgttcgagtggtacgaccagtcgggcctgtcggtggtcatgccggtgggtggccagtcaagcttctactccgactggtaccagcccgcctgcggcaaggccggttgccagacttacaagtgggagaccttcctgaccagcgagctgccggggtggctgcaggccaacaggcacgtcaagcccaccggaagcgccgtcgtcggtctttcgatggctgcttcttcggcgctgacgctggcgatctatcacccccagcagttcgtctacgcgggagcgatgtcgggcctgttggacccctcccaggcgatgggtcccaccctgatcggcctggcgatgggtgacgctggcggctacaaggcctccgacatgtggggcccgaaggaggacccggcgtggcagcgcaacgacccgctgttgaacgtcgggaagctgatcgccaacaacacccgcgtctgggtgtactgcggcaacggcaagccgtcggatctgggtggcaacaacctgccggccaagttcctcgagggcttcgtgcggaccagcaacatcaagttccaagacgcctacaacgccggtggcggccacaacggcgtgttcgacttcccggacagcggtacgcacagctgggagtactggggcgcgcagctcaacgctatgaagcccgacctgcaacgggcactgggtgccacgcccaacaccgggcccgcgccccagggcgcctagtttcttaagttt

SEQ ID NO: 72 - DNA, 21 bp, Influenza virus
gggaatctattcattgctcct

SEQ ID NO: 73 - DNA, 21 bp, Influenza virus
tggggggttattcaccacccg

SEQ ID NO: 74 - DNA, 24 bp, Influenza virus
cattatgaggaatgttcctgttac

SEQ ID NO: 75 - protein, 20 aa, Mycobacterium tuberculosis
SEFAYGSFVRTVSLPVGADE

SEQ ID NO: 76 - DNA, 60 bp, Mycobacterium tuberculosis
tcggaattcgcgtacggttccttcgttcgcacggtgtcgctgccggtaggtgctgacgag

SEQ ID NO: 77 - protein, 22 aa, Artificial Sequence
  Description of Artificial Sequence: Synthetic peptide
GNLFIAPWGVIHHPHYEECSCY

SEQ ID NO: 78 - DNA, 66 bp, Artificial Sequence
  Description of Artificial Sequence: Synthetic oligonucleotide
gggaatctattcattgctccttggggggttattcaccacccgcattatgaggaatgttcctgttac

SEQ ID NO: 79 - DNA, 1008 bp, Artificial Sequence
  Description of Artificial Sequence: Synthetic polynucleotide
tcggaattcgcgtacggttccttcgttcgcacggtgtcgctgccggtaggtgctgacgaggggaatctattcattgctccttggggggttattcaccacccgcattatgaggaatgttcctgttactcccggccgggcttgccggtggagtacctgcaggtgccgtcgccgtcgatgggccgtgacatcaaggtccaattccaaagtggtggtgccaactcgcccgccctgtacctgctcgacggcctgcgcgcgcaggacgacttcagcggctgggacatcaacaccccggcgttcgagtggtacgaccagtcgggcctgtcggtggtcatgccggtgggtggccagtcaagcttctactccgactggtaccagcccgcctgcggcaaggccggttgccagacttacaagtgggagaccttcctgaccagcgagctgccggggtggctgcaggccaacaggcacgtcaagcccaccggaagcgccgtcgtcggtctttcgatggctgcttcttcggcgctgacgctggcgatctatcacccccagcagttcgtctacgcgggagcgatgtcgggcctgttggacccctcccaggcgatgggtcccaccctgatcggcctggcgatgggtgacgctggcggctacaaggcctccgacatgtggggcccgaaggaggacccggcgtggcagcgcaacgacccgctgttgaacgtcgggaagctgatcgccaacaacacccgcgtctgggtgtactgcggcaacggcaagccgtcggatctgggtggcaacaacctgccggccaagttcctcgagggcttcgtgcggaccagcaacatcaagttccaagacgcctacaacgccggtggcggccacaacggcgtgttcgacttcccggacagcggtacgcacagctgggagtactggggcgcgcagctcaacgctatgaagcccgacctgcaacgggcactgggtgccacgcccaacaccgggcccgcgccccagggcgcc

SEQ ID NO: 80 - protein, 10 aa, Artificial Sequence
  Description of Artificial Sequence: Synthetic peptide
CAGAGNFIAP

SEQ ID NO: 81 - protein, 10 aa, Artificial Sequence
  Description of Artificial Sequence: Synthetic peptide
CAGAGNLIAP

SEQ ID NO: 82 - protein, 11 aa, Artificial Sequence
  Description of Artificial Sequence: Synthetic peptide
CAGAGNLFIAP

SEQ ID NO: 83 - protein, 10 aa, Artificial Sequence
  Description of Artificial Sequence: Synthetic peptide
CAGAWGVHHP

SEQ ID NO: 84 - protein, 10 aa, Artificial Sequence
  Description of Artificial Sequence: Synthetic peptide
CAGAWGIHHP

SEQ ID NO: 85 - protein, 11 aa, Artificial Sequence
  Description of Artificial Sequence: Synthetic peptide
CAGAWGVIHHP

SEQ ID NO: 86 - protein, 11 aa, Artificial Sequence
  Description of Artificial Sequence: Synthetic peptide
CAGAWGIVHHP

SEQ ID NO: 87 - protein, 13 aa, Artificial Sequence
  Description of Artificial Sequence: Synthetic peptide
GNLIAPWGVIHHP

SEQ ID NO: 88 - protein, 17 aa, Artificial Sequence
  Description of Artificial Sequence: Synthetic peptide
CAGAGNLIAPWGVIHHP

SEQ ID NO: 89 - protein, 14 aa, Artificial Sequence
  Description of Artificial Sequence: Synthetic peptide
GNLFIAPWGVIHHP

SEQ ID NO: 90 - protein, 18 aa, Artificial Sequence
  Description of Artificial Sequence: Synthetic peptide
CAGAGNLFIAPWGVIHHP

SEQ ID NO: 91 - protein, 8 aa, Artificial Sequence
  Description of Artificial Sequence: Synthetic peptide
HYEECSCY

SEQ ID NO: 92 - protein, 12 aa, Artificial Sequence
  Description of Artificial Sequence: Synthetic peptide
CAGAHYEECSCY

SEQ ID NO: 93 - protein, 22 aa, Artificial Sequence
  Description of Artificial Sequence: Synthetic peptide
GNLFIAPWGVIHHPHYEECSCY

SEQ ID NO: 94 - protein, 26 aa, Artificial Sequence
  Description of Artificial Sequence: Synthetic peptide
CAGAGNLFIAPWGVIHHPHYEECSCY

SEQ ID NO: 95 - protein, 28 aa, Artificial Sequence
  Description of Artificial Sequence: Synthetic peptide
GNLFIAPWGVIHHPGNLFIAPWGVIHHP

SEQ ID NO: 96 - protein, 32 aa, Artificial Sequence
  Description of Artificial Sequence: Synthetic polypeptide
CAGAGNLFIAPWGVIHHPGNLFIAPWGVIHHP

SEQ ID NO: 97 - protein, 22 aa, Artificial Sequence
  Description of Artificial Sequence: Synthetic peptide
HYEECSCYGNLFIAPWGVIHHP

SEQ ID NO: 98 - protein, 22 aa, Artificial Sequence
  Description of Artificial Sequence: Synthetic peptide
GNLFIAPHYEECSCYWGVIHHP

SEQ ID NO: 99 - protein, 39 aa, Artificial Sequence; identical to SEQ ID NO: 47
  Description of Artificial Sequence: Synthetic polypeptide

SEQ ID NO: 100 - protein, 35 aa, Artificial Sequence; identical to SEQ ID NO: 16
  Description of Artificial Sequence: Synthetic polypeptide

SEQ ID NO: 101 - protein, 48 aa, Artificial Sequence; identical to SEQ ID NO: 17
  Description of Artificial Sequence: Synthetic polypeptide

SEQ ID NO: 102 - protein, 52 aa, Artificial Sequence
  Description of Artificial Sequence: Synthetic polypeptide
VTREPYVSCDPKSCINRCFYVELIRGRVTREPYVSCDPQYIKANSKFIGITE

SEQ ID NO: 103 - protein, 18 aa, Artificial Sequence
  Description of Artificial Sequence: Synthetic peptide
DWSGYSGSFVQHPELTGL

SEQ ID NO: 104 - protein, 33 aa, Artificial Sequence; identical to SEQ ID NO: 18
  Description of Artificial Sequence: Synthetic polypeptide

SEQ ID NO: 105 - protein, 16 aa, Artificial Sequence
  Description of Artificial Sequence: Synthetic peptide
KSCINRCFYVELIRGR

SEQ ID NO: 106 - protein, 12 aa, Artificial Sequence
  Description of Artificial Sequence: Synthetic peptide
GNLFIAPRYAFA

SEQ ID NO: 107 - protein, 16 aa, Artificial Sequence
  Description of Artificial Sequence: Synthetic peptide
CAGAGNLFIAPRYAFA

SEQ ID NO: 108 - protein, 11 aa, Artificial Sequence
  Description of Artificial Sequence: Synthetic peptide
GNLVVPRYAFA

SEQ ID NO: 109 - protein, 15 aa, Artificial Sequence
  Description of Artificial Sequence: Synthetic peptide
CAGAGNLVVPRYAFA

SEQ ID NO: 110 - protein, 11 aa, Artificial Sequence
  Description of Artificial Sequence: Synthetic peptide
GNLIAPRYAFA

SEQ ID NO: 111 - protein, 15 aa, Artificial Sequence
  Description of Artificial Sequence: Synthetic peptide
CAGAGNLIAPRYAFA

SEQ ID NO: 112 - protein, 6 aa, Artificial Sequence
  Description of Artificial Sequence: Synthetic peptide
GNLVVP

SEQ ID NO: 113 - protein, 10 aa, Artificial Sequence
  Description of Artificial Sequence: Synthetic peptide
CAGAGNLVVP

SEQ ID NO: 114 - protein, 15 aa, Artificial Sequence
  Description of Artificial Sequence: Synthetic peptide
FVIREPFISCSHLEC

SEQ ID NO: 115 - protein, 19 aa, Artificial Sequence
  Description of Artificial Sequence: Synthetic peptide
CAGAFVIREPFISCSHLEC